European Patent Application EP 4 595 961 A1, published August 6, 2025. Title: Selexipag for use in the treatment and/or prevention of atherosclerosis. Applicant: SORBONNE UNIVERSITE. The sequence listing filed with the application follows.

SEQUENCE LISTING (14 sequences)

SEQ ID NO: 1 - DNA, 22 bp, synthetic construct
  source 1..22: mol_type = other DNA
ctatgcctctggacgcacaact

SEQ ID NO: 2 - DNA, 22 bp, synthetic construct
  source 1..22: mol_type = other DNA
cagatccagacgcatgatggca

SEQ ID NO: 3 - DNA, 23 bp, synthetic construct
  source 1..23: mol_type = other DNA
ccaacgacctgtttgagaacacc

SEQ ID NO: 4 - DNA, 22 bp, synthetic construct
  source 1..22: mol_type = other DNA
atttccgctcctgcttctctgc

SEQ ID NO: 5 - DNA, 20 bp, synthetic construct
  source 1..20: mol_type = other DNA
aaaaccaaggtccagggaac

SEQ ID NO: 6 - DNA, 20 bp, synthetic construct
  source 1..20: mol_type = other DNA
aggtcctgcatgaatccaaa

SEQ ID NO: 7 - DNA, 22 bp, synthetic construct
  source 1..22: mol_type = other DNA
caagtctgggaccaaagcgttc

SEQ ID NO: 8 - DNA, 24 bp, synthetic construct
  source 1..24: mol_type = other DNA
ctttctcagcaaccaaataagcag

SEQ ID NO: 9 - DNA, 20 bp, synthetic construct
  source 1..20: mol_type = other DNA
caggagcccagctatgaact

SEQ ID NO: 10 - DNA, 18 bp, synthetic construct
  source 1..18: mol_type = other DNA
agcaggcaacaccaggag

SEQ ID NO: 11 - DNA, 22 bp, synthetic construct
  source 1..22: mol_type = other DNA
gtgggtcattctcaaggcacca

SEQ ID NO: 12 - DNA, 22 bp, synthetic construct
  source 1..22: mol_type = other DNA
ccatagggctagtacagaaggc

SEQ ID NO: 13 - DNA, 22 bp, synthetic construct
  source 1..22: mol_type = other DNA
tccaggtctggctgaagaatgg

SEQ ID NO: 14 - DNA, 22 bp, synthetic construct
  source 1..22: mol_type = other DNA
ctgctccatctgcttgaagacc